European Patent Application EP 4 548 933 A1, published May 7, 2025. Title: AGENTS FOR IMPROVING COGNITIVE FUNCTION, AND PHARMACEUTICAL COMPOSITIONS FOR TREATING OR PREVENTING COGNITIVE DYSFUNCTION. Applicant: 国立大学法人東北大学. The sequence listing filed with the application follows.

SEQUENCE LISTING (10 sequences)

SEQ ID NO: 1 - DNA, 21 bp, synthetic construct
  source 1..21: mol_type = other DNA
aggtcggtgtgaacggatttg

SEQ ID NO: 2 - DNA, 19 bp, synthetic construct
  source 1..19: mol_type = other DNA
ggggtcgttgatggcaaca

SEQ ID NO: 3 - DNA, 22 bp, synthetic construct
  source 1..22: mol_type = other DNA
gcaactgttcctgaactcaact

SEQ ID NO: 4 - DNA, 21 bp, synthetic construct
  source 1..21: mol_type = other DNA
atcttttggggtccgtcaact

SEQ ID NO: 5 - DNA, 23 bp, synthetic construct
  source 1..23: mol_type = other DNA
ccctcacactcagatcatcttct

SEQ ID NO: 6 - DNA, 19 bp, synthetic construct
  source 1..19: mol_type = other DNA
gctacgacgtgggctacag

SEQ ID NO: 7 - DNA, 21 bp, synthetic construct
  source 1..21: mol_type = other DNA
ccccagctagttgtcatcctg

SEQ ID NO: 8 - DNA, 22 bp, synthetic construct
  source 1..22: mol_type = other DNA
caagtgatttttgtcgcatccg

SEQ ID NO: 9 - DNA, 22 bp, synthetic construct
  source 1..22: mol_type = other DNA
gctggacaacatactgctaacc

SEQ ID NO: 10 - DNA, 21 bp, synthetic construct
  source 1..21: mol_type = other DNA
atttccgataaggcttggcaa